European Patent Specification EP 3 384 054 B1, published November 29, 2023. Title: MULTIPLEX NUCLEIC ACID REFERENCE MATERIALS. Applicant: SERACARE LIFE SCIENCES, INC. The sequence listing filed with the application follows.

SEQUENCE LISTING (40 sequences)

SEQ ID NO: 1 - DNA, 9862 bp, Homo sapiens
ctcgagtactgctcacctggagggccactgacaaccacccttaacccctcctcccagagaccccagttgcaaaccagacctcaggcggctcatagggcaccaccacactatgtcgaaaagtgtttctgtcatccaaatactccacacgcaaatttccttccactcggataagatgctgaggaggggccagacctaagagcaatcagtgaggaatcagaggcctggggaccctgggcaaccagccctgtcgtctctccagccccagctgctcaccatcgctatctgagcagcgctcatggtgggggcagtgcctcacaacctccgtcatgtgctgtgactgcttgtagatggccatggcgcggacgcgggtgccgggcgggggtgtggaatcaacccacagctgcacagggcaggtcttggccagttggcaaaacatcttgttgagggcaggggagtactgtaggaagaggaaggagacagagttgaaagtcagggcacaagtgaacagataaagcaactggaagacggcagcaaagaaacaaacatgcgtaagcacctcctgcaacccactagcgagctagagagagttggcgtctacacctcaggagctcccgggtgggactgagtggctgtggtagagatcccatcctgccaaagtttgtgattccacatttctcttccattgtagagcaaatccatccccacaccctgttcactcctttgctgattggtttcgtaatcgtagctggcatgatgtgcattattgtgatgattctgacctacaaatatttacaggtaaccatttatttgttctctctccagagtgctctaatgactgagacaataattattaaaaggtgatctatttttccctttctccccacagaaacccatgtatgaagtacagtggaaggttgatgaggagataaatggaaacaattatgtttacatagacccaacacaacttccttatgatcacaaatgggagtttcccagaaacaggctgagttttggtcagtatgaaacaggggctttccatgtcacctttttgggtacacataacagtgactttaaggaactccagtggcttcctttgttttgttccacctgaaacaatgagttttctgtgaaattgcgccccttttgataggtttgccatagagaacatcgtaggaaaatgtctctggacaacattgtttttaattcctttattgattttgaaactgggccggccactgctctgcactaccagcaggcctgtggcatgtgacaagctggccctgtgtgcctgtgggtgggcagctgactcccgccagcatctcagcaatccacaggaggttcaggctggagctccagccccttcaaagatgtgtgtggccagttctgtgcccaggagtgtctacagcactcctctggttactgaaagctcagggatagggcctggccttctcctttacccctccttcctagagagttagagtaacttcaatgtctttattccatcttctctttagggtcggattccagttaaatggacggcaattgaatccctttttgatcatatctacaccacgcaaagtgatgtgtaagtgtgggtgttgctctcttggggtggaggttacagaaacacccttatacatgtagtggggccacgacgcccgtctgtgcagcttggccagggaattgcactggccctgagcacctgtctgcagtgctagccctctgcaatgaccccctcactgaggggccttcatgatgtgttcgtgaggcaaatggctgggccaggccgggctgcagttctgaaagctccggtagagcatgagagccgagcaggtggcatcgatacgaaagcctctctaattttgtgacatttgagcaaagacctgaaggtattaacatcatttgctccaaactgaccaaactgttcttattacttataggtttcaggagatgtgttacaaggcttatctagctattcgacagcatgccaatctcttcataaatcttttctcaatgatgcttggctctggaatgccagaactacaatcttttgatgacattgcatacattcgaaagaccctagccttagataaaactgagcaagaggctttggagtatttcatgaaacaaatgaatgatgcacgtcatggtggctggacaacaaaaatggattggatcttccacacaattaaacagcatgcattgaactgaaaagataactgagaaaatgaaagctcactctggattccacactgcactgttaataactctcagcaggcaaagaccgattgcataggaattgcacaatccatgaacagcattagaatttacagcaagaacagaaataaaatactatataatttaaataatgtaaacgcaaacagggtttgatagcacttaaactagttcatttcaaaattaagctttagaataatgcgcaatttggtacctttgttctacaaatattatgtcttagattggttctttcctgtctctgaaaataaagtcttgcaatgaaaataaattattttacaacagttaattagcaatgtaaaatttattgaaaatgtatttgctttttctgtaaatcatctgtgaatccagaggggaaaaatatgacaaagaaagctatataagatattattttattttacagagtaacagactagctagagacaatgaattaagggaaaatgacaaagaacagctcaaagcaatttctacacgagatcctctctctgaaatcactaagcaggagaaagattttctatggagtcacaggtaagtgctaaaatggagattctctgtttctttttctttattacagaaaaaataactgaatttggctgatctcagcatgtttttaccatacctattggaataaataaagcagaatttacatgatttttaaactataaacattgcctttttaaaaacaatggttgtaaattgatatttgtggaaaatcatactacattggtagttggcacattaaatgctttttcttactctgaattcctgatatgactttctttaggattgtttaaaatgcgcgctacgcaggtcagggagtctgaaatcatcaggcatctactcttctctagagctttctctctgttgggagtgggtggagtgagaacctgggagaaggccagccctttatatccaggcagacagctccaagtgccaccatggatcagccagtcttgcaggggtgatgctattcagctacagatggcttgatcctgagtcatttcttccttttccatgcagtgtgtccaccgtgatctggctgctcgcaacgtcctcctggcacaaggaaaaattgtgaagatctgtgactttggcctggccagagtcatcatgcatgattcgaactatgtgtcgaaaggcagtgtacgtcctcacttccctcactggtcaggctcatcctccttcactttaatctctaaagtcaggtgttgcttctagagattcggtgcctgttttttaaaacatcaatagatttcaaggggtcagtacactgccttggcagcagattgcccaggtttgagtgccagctccaccacttacttaatttggatttggggctagatacttgactgttctgcccctctgtctccctgattgtagtgggaggtgataatagtacctatttgcggcgcctaacagtatattatgtaaaataaattccagtattaactttcagtaattaccctagattctcaatgtcaaacaacctaaaaccaactcttcccataattaaaaagctctatcttccctagtgtggtaacctcatttccccataaagattcagaacacaaagatcatcctttcagagaaaataatgctcctagtacctgtagaggttaatatccgcaaatgacttgctattattgatggcaaatacacagaggaagccttcgcctgtcctcatgtattggtctctcatggcactgtactcttctcgtccagctgtatccagtatgtccaacaaacaggtttcaccatctataaccacttgttttctgtaagaatcctgggggtgtggagggtaagggggcagggagggagggaagttcaatttttattaaaaaccacagggaatgcaatgctattgccaaggttaaataagcatctaactattcaagcccatttctgcctatctggtttgtccctcaaattgctaatatataatcacaaacaaaaagtatccaatatcaccctacataaaagaaaacccaccaaattctatatgcctgcagaaaaggtttaaacatgcacagagagtgaacatcatggaccctgacatactcccaaggaaagtaaagttcccatattaatggttacatataacttgaaacccaaggtacatttcagataacttaactttcagcataattatcttgtaataagtactcatgaaaatggtcagagaaacctttatctgtatcaaagaatggtcctgcaccagtaatatgcatattaaaacaagatttacctctattgttggatcatattcgtccacaaaatgattctgaattagctgtatcgtcaaggcactcttgcctacgccatcagctccaactaccacaagtttatattcagtcattttcagcaggccttataataaaaataatgaaaatgtgactatattagaacatgtcacacataaggttaatacactatcaaatactccaccagtaccttttaatacaaactcacctttatatgaaaaattatttcaaaataccttacaaaattcaatcatgaaaattccagttgactgcagacgtgtatcgtaatgaactgtacttcatttacaaactcctccatcgacgcttaagaaaaatgcataaatgctacatagacagttctcggaccgttagtagagatgggatttcaccatgttggccaggttggtgtcaaactcctgacctcatgatccgcccgcctcggcctcccaaagtgctgggattacaggtgtgagccaccgtgcccggcctaatctttgtatttttagtagagacagggtttcaccatgttgtccaggctggtactttgagccttcacaggctgtgggccatggctgtggtttgtgatggttgggaggctgtgtggtgtttgggggtgtgtggtctcccataccctctcagcgtacccttgtccccaggaagcatacgtgatggcatacgtgatggctggtgtgggctccccatatgtctcccgccttctgggcatctgcctgacatccacggtgcagctggtgacacagcttatgccctatggctgcctcttagaccatgtccgggaaaaccgcggacgcctgggctcccaggacctgctgaactggtgtatgcagattgccaaggtatgcacctgggctctttgcaggtctctccggagcaaacccctatgtccacaaggggctaggatggggactcttgctgggcatgtggccaggcccaggccctcccagaaggtctacatgggtgcttcccattaattaatgcacccaggaggggccctctcccactgcatctgtcacttcacagccctgcgtaaacgtccctgtgctaggtcttttgcaggcacagcttttcctccatgagtacgtattttgaaactcaagatcgcattcatgcgtcttcacctggaaggggtccatgtgcccctccttctggccaccatgcgaagccacactgacgtgcctctccctccctccaggaagcctacgtgatggccagcgtggacaacccccacgtgtgccgcctgctgggcatctgcctcacctccaccgtgcagctcatcatgcagctcatgcccttcggctgcctcctggactatgtccgggaacacaaagacaatattggctcccagtacctgctcaactggtgtgtgcagatcgcaaaggtaatcagggaagggagatacggggaggggagataaggagccaggatcctcacatgcggtctgcgctcctgggatagcaagagtttgccatggggatatgtgtgtgcgtgcatgcagcacacacacattcctttattttggattcaatcaagttgatcttcttgtgcacaaatcagtgcctgtcccatctgcatgtggaaacgccggtggactttataacaggctttacaagcttgagattcttttatctaaataatcagtgtgattcgtggagcccaacagctgcagggctgcgggggcgtcacagcccccagcaatatcagccttaggtgcggctccacagccccagtgtccctcaccttcggggtgcatcgctggtaacatccacccagatcactgggcagcatgtggcaccatctcacaattgccagttaacgtcttccttctctctctgtcatagggactctggatcccagaaggtgagaaagttaaaattcccgtcgctatcaagacatctccgaaagccaacaaggaaatcctcgatgtgagtttctgctttgctgtgtgggggtccatggctctgaacctcaggcccaccttttctcatgtctggcagctgctctgctctagaccctgctcatctccacatcctaaatgttcactttctatgtctttccctttctagctctagtgggtataactccctccccttagagacagcactggcctctcccatgctggtatccaccccaaaaggctggaaacaggcaattactggcatctacccagcactagtttgctcttcagtcaaagttaatggtcagcagcgggttacatcttctttcatgcgcctttccattctttggatcagtagtcactaacgttcgccagccataagtcctcgacgtggagaggctcagagcctggcatgaacatgaccctgaattcggatgcagagcttcttcccatgatgatctgtccctcacagcagggtcttctctgtttcagggcatgaactacttggaggaccgtcgcttggtgcaccgcgacctggcagccaggaacgtactggtgaaaacaccgcagcatgtcaagatcacagattttgggcgggccaaactgctgggtgcggaagagaaagaataccatgcagaaggaggcaaagtaaggaggtggctttaggtcagccagcattttcctgacaccagggaccaggctgccttcccactagctgtattgtttaacacatgcaggggaggatgctctccagacattctgggtgagctcgcagcagctgctgctggcagctgggtccagccagggtctcctggtagtgtgagccagagctgctttgggaacagtacttgctgggacagtgaatgaggatgttatccccaggtgatcattagcaaacgtacgtgttaggtggttccctaagggattaggtatttcatcactgagctaaccctggctatcattctgcttttcttggctgtctttcagatttgactttatttctaaaaatatttcaatgggtcatatcacagattctttttttttaaattaaagtaacatttccaatctactaatgctaatactgtttcgtatttatagctgatttgatggagttggacatggccatggaaccagacagaaaagcggctgttagtcactggcagcaacagtcttacctggactctggaatccattctggtgccactgccacagctccttctctgagtggtaaaggcaatcctgaggaagaggatgtggatacctcccaagtcctgtatgagtgggaacagggattttctcagtccttcactcaagaacaagtagctggtaagagtattatttttcattgccttactgaaagtcagaatgcagttttgagaactaaaaagttagtgtataatagtttaaataaaatgttgtggtgaagaaaagagagtaatagcaatgtcacttttaccatttaggatagcaaatacttaggtaaatgctgaactgtggatagtgagtgcctgcaggctgtttataagacatatatttttgtttgaaatacactgaaactggtttcaaaatattcgttttaagggtaaagaaaaaagttaaaaaatctatttacataaaaaataagaacactgatttttgtgaatactgggaactatgaaaatactatagttgagaccttcaatgactttctagtaactcagcagcatctcagggccaaaaatttaatcagtggaaaaatagcctcaattcttaccatccacaaaatggatccagacaactgttcaaactgatgggacccactccatcgagatttctctgtagctagaccaaaatcacctatttttactgtgaggtcttcatgaagaaatatatctgaggtgtagtaagtaaaggaaaacagtagatctcattttcctatcagagcaagcattatgaagagtttaggtaagagatctaatttctataattctgtaatataatattctttaaaacatagtacttcatctttcctcttagagtcaataagtatgtctaaaacaatgattagttctatttagcctatataacctgcttttaagatttttggggcttgaaatgtgttaggatgaggtgagagacgtcgcttgagatcaagattgcagatacagaatccatatttcgtgtatattgctgatattaatcattaaaatcgtttttgacagtttgacagttaaaggcatttcctgtgaaataatactggtatgtatttaaccatgcagatcctcagtttgtggtctgccagctaaaggtgaagatatattcctccaattcaggacccacacgacgggaagacaagttcatgtactttgagttccctcagccgttacctgtgtgtggtgatatcaaagtagagttcttccacaaacagaacaagatgctaaaaaggtttgtactttactttcattgggagaaatatccaaaataaggacagattaaaagctatattttattttatgacatgtaaggaactataatttgttttctattagatctgcaggtgttttgcttactctggcattggtgagacattataagggtaaataatcctgtttgaaggaaaaggccttatggcattgtaacatgagaggaatttttcttaacaaggatggttaactgagaagaaattagcatgggaccaatattttaaaaattttggtctataggtagaaatgagatctgttctgtaccaggtggcaatatcatatggtataactgaataaaaggataaaggaaaaaaaacagcatgtttgaaaaaaaatgtgttgagatggacgcctatttgtaagtttatttgtatttgcctttagctaaatgtgtgtaaatatacagttatacatatatgcatttctcaatttcataccttgcttaatgggtgtagataccaaaagataagaataaaacacatacaagttggaaatttctgggccatgaaaaaaaaaacatgcaaaatcacattattgccaacatgacttacttgatccccataagcatgacaacctatgatgataggttttacccatccactcacaagccgggggatatttttgcagataatggcttctctgaagaccgtgccacccagaatatttcgtatggtgccatttggtgatttccacatttgtttcaacttgaactcctcaaccctcttctcatcaggagtgatagtggcacatttgacgccaacattatgcttctttatagcttctgcagcatccttggtgacttggtcgttggtggcatcacgattctctatgcctaaatcatagcttgaaagagaaaaattagaagcaaagtttttcagacaaatggatagttataacctacaactgcagtgatggcatatagagctcattatgcagaaagcgaaggctctgagtacaccaaaagcggccgc

SEQ ID NO: 2 - DNA, 9179 bp, Homo sapiens
ctcaaactcctagcctcgagtcatccacccgcctcgtcctcccggagtgcttggattacagcatgagccactgcgcccggcccccattttagttttgatggacatttgggtaattttcttttttggctattctaaataatgctgcaattactgttaattttcaccttgtaaaaaccattttcaaatctcaagagattaacctttagttttcttggtttggattgggaaggaacaccaaggaaaatgagggacttcagaatttattttcattttgcatttgttttttaaaatctttagaactggatccagtggtatagaaatcttcgatttttaaattcttaattttaggttgcagtttcatcactgtctgcggtaatcaagtttttagaactcttatcagatgattccaactttggacagtttgaactgactacttttgacttcagccagtatatgaaattggatattgcagcagtcagagcccttaacctttttcaggttaaaaaaaaaaaaaaaaaaaaaaaaaagggttaaaaatgttgaatggttaaaaaatgttttcattgacatatactgaagaagcttataaaggagctaaaatattttgaaatattattatacttggattagataactagctttaaatggctgtatttttctctcccctcctccactccactttttaacttttttttttttaagtcagagtctcacttgttccctaggccagagtgcagtggcacaatctcagcccactctaacctccacctcccaagtagttgggattacagttgcctgccaccatgcctggttaatttttatatttttagtagggttgcggggacagggtttcaccatgttggccaggttggtctcaaacttctgaccttaggtgatcctcccacctcggcttcccaaagtgctgggattacaggcttgagccatcgtgcccagcctactttttacttttttagagactgggcttggtggagtgaagtggccctcctgagaagctgggattacaagcacgcgccaccatgctgggctaatttttgtatttttagtagagacggggtttctccatgttggtcaggctggtctcgaactcctgacctcaggcaatccaccgacctcaggtgatccacccgcctcagcctcccaaagttctggggttacaggcgtgagccaccacgcccggctgtcttcaatcttaaataaggattccatttaaatattttgtaaaaggacacagatcacagttttactcaggggaatataattgttatagcaggaattgtgccattgcgctattccaaacagtgtaaaagaacattaataaattgaattctaactacatttgtccctaaggagttgttcgttttccacttgtatttccattttaattatcattatttggatgtttcataggatactttggatatgtttcacgtagtacacattgcttctagtacacattttaatatttttaataaaactgttataatgaagagtataccaaaaataaaacagaatatgaagaagcccaggatgccattgttaaagaaattgtcaatatttcttcaggtaaacttaatagaactaataatgttctgaatgtcacctggcttttggtaacagaagaaaaatcatgatatttgaagtgtgttttgttattttcgcaagccattacattctgactatttaatatgttaggtttcctatataaaataaggcatggtatgttacagtaggacacataactggaagttactcttgcacatagaaacaaaaaatggcagaaaagcacaaaacttactatagttgtaacagggaaaggaaacactagggcctacaacgtactaatgtcttgggtcatctatgggctcatgaggctctaggttatggaagtaaataccactgaaaagcaaatattaattacacatgaggcaagcctttttgagttctgtatgtcattttgtagattttgagttcattctagtggcagggtacacagacttacagtgtgctggaaggtgatccctctgagaactacagtaagtatcttcttagcctcaaagaaaaagaggaagattcttctggccatactcgtgcatatggtgtgtgctttgttgatacttcactgggaaagtttttcataggtcagttttcagatgatcgccattgttcgagatttaggactctagtggcacactatcccccagtacaagttttatttgaaaaaggaaatctctcaaaggaaactaaaacaattctaaagagttcattgtcctgttctcttcaggaaggtctgatacccggctcccagttttgggatgcatccaaaactttgagaactctccttgaggaagaatattttagggaaaagctaagtgatggcattggggtgatgttaccccaggtgcttaaaggtatgacttcagagtctgattccattgggttgacaccaggagagaaaagtgaattggccctctctgctctaggtcttctacctcaaaaatgtcttctacctcaaaaaatgccttattgatcaggagcttttatcaatggctaattttgaagaatatattcccttggattctgacacagtcagcactacaagatctggtgctatcttcaccaaagcctatcaacgaatggtgctagatgcagtgacattaaacaacttggagatttttctgaatggaacaaatggttctactgaaggaaccctactagagagggttgatacttgccatactcctttttgcggctcctaaagcaatggctttgtgccccactctgtaaccattatgctattaatgatcgtctagatgccatagaagacctcatggttgtgcctgacaaaatctccgaagttgtagagcttctaaagaagcttccagatcttgagaggctactcagtaaaattcataatgttgggtctcccctgaagagtcagaaccacccagacagcagggctataatgtatgaagaaactacatacagcaagaagaagattattgattttctttctgctctggaaggattcaaagtaatgtgtaaaattatagggatcatggaagaagttgctgataaaagttttaagtctaaaatccttaagcaggtcatctctctgcagacaaaaaatcctgaaggtcgttttcctgatttgactgtagaattgaaccgatgggatacagcctttgaccatgaaaaggctcgaaagactggacttattactcccaaagcaggctttgactctgattatgaccaagctcttgctgacataagagaaaatgaacagagcctcctggaatacctagagaaacagcgcaacagaattggctgtaggaccatagtctattgggggattggtaggaaccgttaccagctggaaattcctgagaatttcaccactcgcaatttgccagaagaatacgagttgaaatctaccaagaagggctgtaaacgatactggaccaaaactattgaaaagaagttggctaatctcataaatgctgaagaacggagggatgtatcattgaaggactgcatgcggcgactgttctataactttgataaaaattacaaggactggcagtctgctgtagagtgtatcggcagtgttgggtaagactttgaacaagcttgttctcaggctttgataagtagtgctgtttgccagctgtatattatccctaaaaataagtaataaggtatatatggtacatattttgacatgcatatacatatttgcatcctgactaggctgcccacagcaatttaagttacttgaaactcgcttttatcttagtagccctttggcctttcttcagtttttttttttttttttttttttttgagacatggtcttgctctgttgcccaggctagaatatggtgacacaaccatggctactgcagcctcgacctcccaggcttaagtgatctttccacctcagcctcccaagtagctgagattacagatatgcaccaccatgcatggctaatatttaaatgtttgtagagagatggggtctcactgtgttgccaggactggtcttgaactcctgggctcaagtgatcctcctgcctcggcttcccaaagtgctgaggttacagcagtgctttgggaggtcaaggcagccagatcatttgagatcaggagttcgagaccagcatggccagcatagtgaagccccatctctactaaaaatacaagaaaaaattaaccaagcatggtggcgcatacctgtaatcccagccactctggaggctgagacatgaaaattgcttgaacccgggaggcggaggttgcagtgagctgagatctcgccactgcacttcagcctgggtgacagagcaagactctgtctcaaaggaggttgcagtgagctgagatctcgccactgcacttcagcctgggtgacagagcaagactctgtctcaaaaaaaaaaaaaacaaaaaccaagaaaagaaaaaaaaactcttctaagaggatttttttttcctggattaaatcaagaaaatgggaattcaaagagatttggaaaaatgagtaacatgattatttactcatctttttggtatctaacagaaagaagatctggatattgtatgtatgtaaggactagtaaactgcagtcctttgaggatttagccagtatttctacctatggctttcgaggtgaggtaagctaaagattcaagaaatgtgtaaaatatcctcctgtgatgacattgtctgtcatttgttagtatgtatttctcaacatagataaataaggtttggtaccttttacttgttaaatgtatgcaaatctgagcaaacttaatgaactttaactttcaaagactgagaattgttcataaataaactattttacctgcagagacctctgatatatgtttcttgatggaagtacccagtaccacctatgaagttttcttgtcaaaaaatcaaatgtgaatctgatcattacttagatctaagtaccaatatatgaaaaatataggagacaaggaagcatggtaaatgatactgagattgggagactacatggaaaaagacttgttcccttcaacagatagacagcagggaaaaaagaatagagaaaggagtaaagaacattcaatttaacttactctccatcctcacccgcccagctttggttatgaggcagtagaaagaaatgatctgcctgtggttttctagaaatacgaaagttgagtccttaaggctacacagaaagaaagtacctccccagggcttcacccttcccatcctttcagcaggctttttgtctgtcgtatcttctctgttgaaatggccattgacaagaggaggaaaggggttttgttgtggattgttcaggcacttcctttggggtatatgggggatgagtgttacatttatggtttctcacctgccattctgatagtggattcttgggaattcaggcttcatttggatgctccgttaaagcttgctccttcatgttcttgcttcttcctaggagccagcaccgctctttgaccttgccatgcttgccttagatagtccagagagtggctggacagaggaagatggtcccaaagaaggacttgctgaatacattgttgagtttctgaagaaggctgagatgcttgcagactatttctctttggaaattgatgaggtgtgacagccattcttatacttctgttgtattcttcaaataaaatttccagccgggtgcggtggctcatggctgtaatcccagcactttgggaggctgaggtgggcagataacttggggtcaggagttcaaaaccagctggccaacatgatgaaaccccgtctctactaaaaaaatagaaaaattagccaggcgtggtggcgggtacctgtaatccaagctgctcaggaggctgaggcagaagaatcacttaaacccaagaggtagaagttgcagtgagccgagattgcaccactgcactctagcctaggcgacagcgagactgcgtctcaaaaaaaaaaaaaaagaacgttccaaggtcaggactaggcctcccctcagaagcagcaagtgacatatgtgacatcctctccactccctatttgcatttctaggttatataactgtactacttctgtcgcccaggttggagtgcagtggtatgaacttggctcactgcaagttccgccttctgggttcacgccattctcctgcctcagcctcccgagtagctgggactataggcgcccgacaccacgcccggctaatttttttgtatttttagtagagacgggctttcaccatgttagccaggatggtctcgatctcctgaactcgtgatccgcccgcctcagcttcccaaagtgctgggattagaggcttgagccaccatgcccggccaagaatactgcttaacagaggtaacaaaagagcaataattatgagttcaaggtcacagagaacgcagacgacacagatgctcagctacgacgctgcacgtagctctctgtgtaaaatgacccctggcaatcacaaaggcgtttacaaccttgaccaaatcaggagctgggctgagaccttcctcgactgcaagcttgagcagctgagctgacagccaggctttctttacttacccacttccggcaggctctggaggcaaacatctgcttgactcgggaaggccggcacatgaccccagggctgtcgctcagcatgaagatcagttcatcgacgtcctggggtccgaaggtccagtttttactagttggcaaggaaatcagtttagccctttcagtgactggagctaaaagaatacaattttgagaaaaatccatgacttgacaaacacgtttcacttgaaagctacttaggatgaacatctgaggccgggcgtggtggctcacgcctgtaatccctgcactttgggaggctgaggccagcggatcatgaggtcaggagatacagaccatcctggctaacatggtgaaaccccgtctctactaaaaaatagaaaaaattagctgggtgtggtggcaggcacctgtagtcccagctactcgggaggctgaggcaggagaatggtgtgaacctgggaggcggagcttgcagtgagccgagatcggcaccactgcgctccagcctgggcgacagagcaagactccatctcagaaaaaaaaaaagtgaacacctgaaagagaggaaactcacaaaatgctttttggaggaactttttaatcttttataaaattaaaaaaaactggtctatatgacctgaaagattattcccagctctaaaaagacaagaatctatagttctgatttttttttttttttgagacagagtttcactcttgttgcccaggctggagtgcagtgacgtgatctcggctcactgcaacctccacctcccgggttcaagcgattctcccacctcagcctcctgagtagctgggattacaggcacccgccaccacgcccggctactttttgtattttcagtagagatggggtttcaccatgttagccaggctggtctcaaactcctgacctcaggcgatctgcccgccttggcctcccagagtgctgggattacagacgtgagccaccacacccagccgctatagttctaattaataacttaccattttcatcgataacaaaatcaaagccattctaaatatttccagattttctatcagaacagcttcattaacagcagttaagttgagagtctgaggtctgaaaaacacaaaaatgattcaaaccatatcctgaagtcaaacatttagctttacagcagaaatgaaatgaaaacaacaatactgtattttgaattcatgtcaaaataacaacacaaataacaacactactcagctaagtgtcacaaaacttcctgagaagttccttttaattttctctttcttaaagttctttttagaagttaaagtagctacaggccaggtgcggtggctcacgcctgtaatctcagcactttaggagcccgaggcaggcagatctcttgaggccaggagtttgagaccggcctggtcaacacagcgaaacactctctctactaaaaatataaaaattaggccaggcatggtggcgcacgcctgtagtcccagctacttgggaggcttaggcatgagattcgtttgaacccaggagggagctgtcacccaggctggagtgcagtggcataatctcggcttactgcaagctccatctcccaggttcaagtgatcctcctgcctcagcctcccatgtagctgggattacaggcgtggaacaccatgcctggttattttttgtattttagtagagacggggttttgtcatgttggccaggctggtctcgaactcctggcctcaggcaatccacccgcctcggcctcccaaagtgctgggattacaggcatgagccactgcgcccggacagaaaagtcttcagttgaaacatctgaagctgggggccatctgcggtagacttctgtaaatgcacaaaataagataatgttaaagccatgtttctcaaagtcccgagctccacgtaaactgcctattatcagaaaaaagttatcaattaaaagtcaaaggcataaagaacaaactaacacaaaaaaattttaaatacctttgctgggtcacaaggccgccggttgataaagaaaaactgtctgttgaactccttccaactccatgcgtgcattgtgaaatgaaacctgagatgctattcaacattaatatggtaagggcaggattccagagtgaaagggattagaaatacgatcacatggcacattcttaaagtgaaatgaaaacaaaacaccaggtgacatgctgataaggatcactattgcagttcacgggtatctgtgctccaaatcttgatgagtcatcaaagaaccaaaccttctggaatattctaaagctcctacagtcaaccaatgcaccacaggtgatgcagtgcgtccaaaactgatgtgttgcagctctccttacccttcctgataaatcctcagcctctgtaagtgggtctcgcttcaaatgcattctcagaacctccgtgctgccacccctggtttgtcaatgaagtctaaccacttgtgctcagaattttgcccacattccctcccctttcaaaacctcccgggtaggacgcttatatctcatggcggccgc

SEQ ID NO: 3 - DNA, 9832 bp, Homo sapiens
caggtatctgtgaattggaggctaagtagtcccagcacatcttacatttctttaagactccctttttatcccaaacgttcgtaaattttgtatctgataaagagcatacttccatctaatacaaatatgttccccccttcagatcttctcagcattcgagagatctgtacgcgcgtggctcctcattcctcttccttggcttcccaagcccccagggcgtcgccaggaggaggtctgtgattacaaaccccttctgaaaactccccaggaagcctcccctttttccggagaatcgaagcgctacctgattccaattcccctgcaaacttcgtcctccagagtcgcccgccatcccctgctcccgctgcagaccctctacccacctggatcggcctccgaccgtaactattcggtgcgttgggcagcgcccccgcctccagcagcgcccgcacctcctctacccgaccccgggccgcggccgtggccagccagtcagccgaaggctccatgctgctccccgccgccggctccatgctgctccccgccgccggctccatgctgctccccgccgcccgctgcctgctctccccctctccgcagccgccgagcgcacgcggtccgccccaccctctggtgaccagccagcccctcctctttcttcctccggtgctggcggaagagccccctccgaccctgtccctcaaatcctctggagggaccgcggtatctttccaggcaaggggacgccgtgagcgagtgctcggaggaggtgctattaactccgagcacttagcgaatgtggcacccctgaagtcgccccaggttgggtctcccccgggggcaccagccggaagcagccctcgccagagccagcgttggcaaggaaggaggactgggctcctccccacctgccccccacaccgccctccggcctccctgctcccagccgcgctcccccgcctgccagcaaaggcgtgtttgagtgcgttcactctgttaaaaagaaatccgcccccgccccgtttccttcctccgcgatacaaccttcctaactgccaaattgaatcggggtgttttttgttctgattgctttttattccaatatcttaaatggtcacagggttatttcagtgaagagcagttaagagccttgaataatcacaggcaaatgttgaatgataagaaacaagctcagatccagttggaaattaggaaggccatggaatctgctgaacaaaaggaacaaggtttatcaagggatgtcacaaccgtgtggaagttgcgtattgtaagctattcaaaaaaagaaaaagattcaggtaagtatgtaaatgctttgtttttatcagttttattaacttaaaaaatgaccttactaacaaaatgattataaatccagataaagtataaagttagtttatatcagagaagcaaaatccactactaatgcccacaaagagataatataaaagaggatctgtatttattttgaaacaaacatttaaatgataatcacttcttccattgcatctttctcatctttctccaaacagttatactgagtatttggcgtcagtatcaacaactaccggtacaaacctttcattgtaatttttcagttttgataagtgcttgttagtttatggaatctccatatgttgaatttttgttttgttttctgtaggtttcagatgaaattttatttcagatttaccagccacgggagccccttcacttcagcaaatttttagatccagactttcagccatcttgttctgaggtggacctaataggatttgtcgtttctgttgtgaaaaaaacaggtaatgcacaatatagttaattttttttattgattcttttaaaaaacattgtcttttaaaatctcttatgattagttggagctaccagttggcaaatttgctagctaactagtgatctgaaagtaagcctctttgaacctctgatttttcatgaaaagcaattctctcaattctatattatttcaagggtaacaagttacatcctagtctgtgtacttaattttatagaaattgtccttaattttattttctaaaaacatcagggaattcatttaaagtaaatagctgcaaagaccacattggaaagtcaatgccaaatgtcctagaagatgaagtatatgaaacagttgtagatacctctgaagaagatagtttttcattatgtttttctaaatgtagaacaaaaaatctacaaaaagtaagaactagcaagactaggaaaaaaattttccatgaagcaaacgctgatgaatgtgaaaaatctaaaaaccaagtgaaagaaaaatactcatttgtatctgaagtggaaccaaatgatactgatccattagattcaaatgtagcaaatcagaagccctttgagagtggaagtgacaaaatctccaaggaagttgtaccgtctttggcctgtgaatggtctcaactaaccctttcaggtctaaatggagcccagatggagaaaatacccctattgcatatttcttcatgtgaccaaaatatttcagaaaaagacctattagacacagagaacaaaagaaagattttcttacttcagagaattctttgccacgtatttctagcctaccaaaatcagagaagccattaaatgaggaaacagtggtaaataagagagatgaagagcagcatcttgaatctcatacagactgcattcttgcagtaaagcaggcaatatctggaacttctccagtggcttcttcatttcagggtatcaaaaagtctatattcagaataagagaatcacctaaagagactttcaatgcaagtttttcaggtcatatgactgatccaaactttaaaaaagaaactgaagcctctgaaagtggactggaaatacatactgtttgctcacagaaggaggactccttatgtccaaatttaattgataatggaagctggccagccaccaccacacagaattctgtagctttgaagaatgcaggtttaatatccactttgaaaaagaaaacaaataagtttatttatgctatacatgatgaaacatcttataaaggaaaaaaaaataccgaaagaccaaaaatcagaactaattaactgttcagcccagtttgaagcaaatgcttttgaagcaccacttacatttgcaaatgctgattcaggtacctctgtctttttttttttgtaaatagtacatatagttttatagatgacgattccttctgtgtttttttctgctttttaaaatcttcatatcttatatttaatcttaggcatcatctgtatacatgattgtttaggtctttaattaccagtgtttagaatcaggtcactcaaacatggtagataagtttgcatagtttgtgtatatccatcactcttgagacagttttattttaagttccggggtacatgtgcaggatgtgcaggtttgttacataagtaaacgtatgccatgttggtttgctgcacctgtcaacccttcacctgagtattaagcccagcatgcattagctatttttcctggtgctctccttccccccacacacccccacctcctgacagacataggtgttttcatgaactttatgttcatgtgtattttactattattagaggtctatcttcagagaggagtacaagaaatgggattactgggtgcaaaggtaaatggatatgtgtctttgctaggtattgccaaatttatctccagaaatcttgcacaaatctgtactcctgttagcaatgtgtgcgtatacctgcttccacatgacctcagtaaaagaatgtgttgtcatattggtattgaaattttagcactgtaagcaacaggtcattttggaaaacctgagctttcgccaaattcagctattttgatttgcttttattattagcatataccaaaataaataggcatattagagtttcctttcttgcatcttaaaattcatctaacacatctataataacattcttttcttttttttccattctaggacttgcccctttcgtctatttgtcagacgaatgttacaatttactggcaataaagttttggatagaccttaatgaggacattatttttttttttttttttttttttttttttttttttttttttgagacggagtctcgctctgtcgcccaggccggactgtggactgcagtggcgcaatctcggctcactgcaagctccgcttcccgggttcacgccattctcctgcctcagcctcccgagtagctgggactacaggcgcccgccaccgcgcccggctaattttttgtatttttagtagagacggggtttcaccttgttagccaggatggtctcgatctcctgacctcatgatccacccgcctcggcctcccaaagtgctgggattacaggcgtgagccaccgcgcccggccaatgaggacattattaagcctcatatgttaattgctgcaagcaacctccagtggcgaccagaatccaaatcaggccttcttactttatttgctggagatttttctgtgttttctgctagtccaaaagagggccactttcaagagacattcaacaaaatgaaaaatactgttgaggtaaggttacttttcagcatcaccacacattttggtatttttctattttgacagtccagtatcaaggaaatagcttttatacaaattggatagttgaggtagtatgtgaggtaaagtttaatcatatattaattgcccatgaacctcaggagatgggggaatggggaaatgacagcaactagaaagagaagaatgacttgaagggaaatgagttaggagaaattgtgagaaggatgttcagaaatgcagactttgtaagcaaactggaaattggttacaagaataatatgagttatctgtggtttgcagcagtcagcagtgtgattgaggatcacaaggtcaggggttcaagaccagcctgggcaagatgagttttcagtgagctgagatcgcaccactgcactctggcctgggcaatggagtgagactccgtcttgggaaaaaaaaaaagagagagagagagcaagagagagagagagaaagacaccccagtgaagtgaaaagagcaaagtctttagattctcatctgcttaaagtcccagctcttccacttatcagctaagatctgaacccgagacgggaatccaaattacacagcctctctaaatctcttagttttatcattcataaagtagagacaatacttatttatgtggttgggatggaagagtgaaaaaagaacctgtgtgaaagtatctagcactgtgtatgtatgtaataagtcttacaaaatgaagcggcccatctctgcaaaggggagtggaatacagagtggtggggtgagatttttgtcaacttgagggagggagctttacctttctgtcctggggattctcttgctcgctttggaccttggtggtttcttccattgaccacatctcctctgacttcaaaatcatgctgaaagaaaccaaacacaacccatcaggataagagaaagagaagcttccttcaatggaagtggagcagacacgtcatatttaaggcattcaggccaggcgcagtggctcacccctgtaatcctagcactttgggagactgaggcaggcagatcacttgaggtcaggagttcgacaccagtctgaccaacatggtgaaacctcatctctactaaaaatacaaaaaattagttgggcgtggtggcaggcacctgtaatcccagctacttgggaggctgaggcaggagaatcttttgaatgcaggaggtggaggttgcagtgagctgagatggtgccactgcactccagcctgggtaacagagcgagactccatctcgcatctcaaaaaattaaaaataaaattaaaaaaaaaaaaattaggccgggtgtgcctcccacagtgttaggattacaggcatgagccactgcacccgattttttttttcttttgatggagttttgctcttgttgcccaggttagagtgcaatgatgcgatctcagctcactgcaacccccgcctcccaggttcaagtgattctcctgcctcagcctcccgagtagctggaattacaggcaagtgccaccaagcccggctaattttgtatttttagtagaaacggggtttctccatgttggtcaggctggtcttgaactcccgacatcaggtgatccaagcgcctcagcctcccaaagcgctgggattataggtatgagccacagtgcaggcctgcataattcttgatgatcctcattatcatggaaaatttgtgcattgttaaggaaagtggtgcattgatggaaggaagcaaatacatttttaactatatgactgaatgaatatctctggttagtttgtaacatcaagtacttacctcattcagcatttttctttaatagactgggtcacccctaaagagatcatagaaaagacaggttacatacagcagaagaacgtgctcttttcacggagatagagaggtcagcgattcacaaaagagcacaggaagaatgacagaggagaggtccttccctctaaagccacagccctttaataaggcttgtagcagcagtttccttctggagacagagttgatgtttaatttaaacattataagtttgcctgctgcacatggattcctgccgactattaaataaatccctagctcatatgctaacattgctaggagcagattaggtcctattagttataaaagagacccattttcccagcatcaccagcttatctgaacaaagtgatattaaagataaaagtagtttagtattacaattaaagaccttttggtaactcagactcagcatcagcaaaaaccttaggtgttaaacgttaggtgtaaaaatgcaattctgaggtgttaaagggaggaggggactatgaaaagcaccttaggaggaacatgtttcaagtttaagaagcagttcctttaactatacttggaaatttgtaaaatgtgctccccaaaagcataaacatttagctcacttctataaatagactggggcaaacacaaaaacctggttccaatacctaagtttgaatccatgctttgctcttcttgattattttcttccaagcccgttcctctttcttcatcatctgaaaccaattccttgtcactcagaccaactccctggctttcagactgatgcctcatttgtttggaagaaccaatcaagaaaggatcctgggtgtttgtatttgcagtcaagtcttccaattcactgcactgtgaagaaaacaagctagcagaacattttgtttcctcactaaggtgatgttcctgagatgcctttgccaatattacctggttactgcagtcatttaagctattcttcaatgataataaattctcctctgtgttcttagacactcggtagcaacggtgctatgcctagtagactgagaaggtatattgtttactttaccaaataacaagtgttggaagcagggaagctcttcatcctcactagataagttctcttctgaggactctaatttcttggcccctcttcggtaaccctgagccaaatgtgtatgggtgaaagggctaggactcctgctaagctctcctttctggacgcttttgctaaaaacagcagaactttccttaatgtcattttcagcaaaactttatttcaccatcatctaacaggtcatcaggtgtctcagaacaaacctgagatgcatgactacttcccataggctgttctaagttatctgaaatcagatatggagagaaatctgtattaacagtctgaactacttcttcatattcttgcttttttatttcaggatgcttacaattacttccaggaagactttgtttatagacctcaggttgcaaaacccctaatctaagcatagcattcaattttggccctctgtttctacctagttctgcttgaatgttttcatcactggaacctatttcattaatactggagcccacttcattagtactggaacctacttcattaatattgcttgagctggctcctttaaaaacattttctccggctaattgtgctcactgtacttggaatgttctcatttcccatttctctttcaggtgacattgaatgttcctcaaagttttcctctagcagatttttcttacatttagttttaacaaatgacttgatgggaaaaagtggtggtatacgatatgggttttgtaaaagtccatgtttatttggagtaatgagtccagtttcgttgcctctgaactgagatgatagacaaaacctagagcctcctttgagtacatttggcattatcaactggcttatctttctgaccaaccacaggaaagcctgcagtgatattaactgtctgtacaggcttgatattagactcattctttccttgattttcttccttttgttcacattcaaaagtgacttttggactttgtttctttaaggacccagagtgggcagagaatgttgcacattcctcttctgcatttcctggatttgaaaacggagcaaatgactggcgctttgaaaccttgaatgtattctgcaaatactgagcatcaagttcactttcttccatttctatgcttgtttcccgactgtggttaacttcatgtcccaatggatacttaaagccttctgtgtcatttctattatctttggaacaaccatgaattagtcccttggggttttcaaatgctgcacactgactcacacatttatttggttctgtttttgccttccctagagtgctaacttccagtaacgagatactttcctgagtgtttagtggagagggggtttcaccatgttggccaggatggtctcgatctcctgacctcgtgatcctaccaccttggcctcccaaagtgctgggattacaggcataagccaccgccctcggcctcatccatgattttattttgccatttcaagtgatggagcttgttttagagctggaagaaaagccaaaatgccagttaatctaaactagattcctgccccagtgcagaaccaatcaagacagagtccctgtctttcccggaccacaggatttgtgttgaaaaggagaggagtgggagaggcagagtggatggagaacaaggaatcattttctatatttttaaagttcttcagttaagaaaatcagcaattacaatagcctaatcttactagacatgtcttttcttccctagtatgtaaggtcaattctgttcatttgcataggagataatcataggaatcccaaattaatacactcttgtgctgacttaccagatgggacactaagattttctgcatagcattaatgacattttgtacttcttcaacgcgaagagcagataaatccatttctttctgttccaatgaactttaacacattagaaaaacatatatatatatctttttaaaaggtttataaaatgacaacttcattttatcattttaaaataaagtaaatttaagatttggaaggttttagaataatacaaaccaaagaactaatgacaacgtcctttatttttaaagattctagaagttgctttttgtaattagacaacataaattctgaattttttcacatattgctgccaaccccttgggtcttttcctttctccaagaaagagaaagctacagaggagtgactgaccgggtaggtggtggtagccttagctttctccaatgtttctggttgttttctttttcttgcataaaaccaaaatcaacaacgaccaaaccaacaccaatcaaggcctccccgcccctaacctttcccagtgacctggcggccgc

SEQ ID NO: 4 - DNA, 10029 bp, Artificial Sequence
  Description of Artificial Sequence: Synthetic polynucleotide
gcggccgcgggtgtggcgtgaatccctgtggagggcgtgtgggcccatgggcgctggtgcgcacgtgtctgggtgcatgtgggcatgtgaaaacacgtgtgcctgtgtgtgccatgtttgcctgtgatggtgcagtgcacataaggaacctcaagtgtctgaggggtggtgatgctcaccaggcccgtatgaccctctcagtaccctctggagcggtcacctcagcatcgtcattttagagatgagaaggatgaggtttaggctgtcaaaggcccaaggtcacagaggccttgagcccaggtttgcctgctcccctacagggctaggtggggtgggggctgaggggtccaagccctaaagcctcatgtgcccccccagccaggctcaccctgcacaatgagctcagccagcgcctggcccccgctagtgcacagtgcatagtgccccgcgtcctccagcatggcctcgttgatgatcaggtggtgtctctgcccgtccttcttgaaccagtatttgaaggtctcctcccgggtcagctccaccccgtccttcagcctagccgggtgggtgggtggcaagtgctgtggcctcttctgggcagatgcccccaacacccatgccccgtgcttctggaactcaccatttgacttgcgccccctcctccgatacttcacactcaaactccacccgctgccccaccatcaccagctggtcctccaaggggcgcgtgatgagcacagggggctctgtccaggcagggtgagcatgagggttggctcccctgaggccatctcctccccaggttcccacatcctcaggtcccaggcccacctttcacaaagagctccgtgctacacttctcgccacccaccacgcactggtaggctgcgtcgtccgccaatgagcactggctgatggtcagggtacgcttggcaccgatggactcaaagatgtacctgggtgggggccgcagggaagtggcaggaaagctgcggacacccctccgggctgtttcctcatctgtaaaatgcggctgagtatccccagtcgaggatgaaaggagactgtggatgtgagtgtctagcatggctgcctgcagagcacctgctattattggaggtttttaactggggagggggcggggggcaggaccaggccaggcaggctcaccgataggcatgaagggctgggaggcagggctgggcctggacatgccgatggcgttgaccgcgtagacgcgcatctcgtacaccacgccctcgatcatgcgccgcgcttcatgactcagctcctgaatcaggtcgaagttcagccgcatccaccggtagctcttcttcttcttgcgctccaggatgtagcctggctcaggggaggtggcagctctggtctggaacccaggcatccccacaccaccttccctcggatctgtttggcgccctcacacctccatccggtgcccttgcactcacccaggatgggctgcccgccatcgtaggcaggcggctcccacctgtactgtgcaggagtcctctcccacgttgctgatcttgggggccgcaggtgcgtctggcacgtctggatggggtgggatggacccacatcagccctgccccgctcagggccttgagtaacgttgctcgtccccttcccactccaactaaccgccacaggctgcccccaccacccccagatccaaagagatctttctagaatgcatttctttcttcttttcctttttttttttttttttttagtgatatggagtctcactgtgttgtccaggctgggtctcaacaggatgcatttctgatcatgtcgccagccctccgtcaaccctttaaggcttctcactgcccatattcacccctgtcctggctctgatcctcccaaccccacccagtcctctcctgacatgtttcattcattctccacacccaaaaggccctttccctcctccacccctttgtacacagtttcctctgcctgggatgcctttcctcaccatcttctatggctgccccaggaccaagggccagggctcagccactgacttgtgccctgggtgtcgggtggtacatacctggccatccccaggagccagcctggtcactgaggcactgcagaagaggaggccatgtcactgtgtcctcccagccttctggaagctattgcccatctgggcgtggcagggtccgtgcccttgcagccagggcaggtgcttggccgaggacaacggagcaaagcccagggtccccactgccgcccgctcttcccatctcccaggccctggccccgagggctcctcacctcgcacctccaggcggcactcacaccgtgcctcgccctgtaagttggtggccctgcagacatagatgcccccgtcaaaggggcagggctttctaatctccagagtcaacactccctgcttgctgaacatgcggaagcgggcgtcttctcccaggtccaggccattcttgaaccaggaaatcttgggctataaataaggtaaagagaggggacctggcagggacccagggagacacatctgtgtttctactcggggggtcccacgagagtccctgactatgcccaaggctggaaacaaacatggaaccaagagtgagtaccatggccctgcccagggggaggaacccggtccatacaccccaaggtggagagaaagcaggggagacaggctggggagaggactgctcaacgtcggggcctgtgagccctgcctcctggtcggcctggaccagcgcctaaagttccctaccttggggctaccccggacagcacagcagagcatagcagtgtagcccgcgatgaccgagcggttcaccaggggctgggtgaagcttggggcctcggagaagtccagggccttatagttgggtggctcataggtgatgcctgttggtgacaggacttggtaccgagagggccacacaaagctaggcccctctccctgttcccacagcctccctgccccagcccctggttggaagaatgagggcagaggggttatgggactggcccaagttcactaagctgatcaagaacagagccaggtcttgaacccaggtccctgagcctctgtctcctaattagccaaaaatggattaacaatttgaatatgtctcattgggggattaagtggttctgcaggtaaatttaaagttgaactaagattctgtcttggacaaccagctatccaaggggttgtagggccactgatgaggtaatgtccatcagagtgccttacacatcaccctcattacacactgcaagtgcaaggtagcgctgagagggaggtaccctgggaggcctcatgcgggatgggaggagaagaatgtggtttggaaaccactgtggtggtaggtagggagatgtcctaggaggtcctgttcccagggcggtgtatgcccagcagtgggttggcctgagtttgtggcctcacctggagactttgtctcattagggatgatacaacgtacaaagtggggatgggtggagtgcaagttggtcatcagcttgttcagattttcctgtggccaaaaatgcaatagagaaaagtaaagaaaatgccagaaagagatgcaggaagaagagaggagaagaaggaaggaaaagagagatggagagaattcgagaagtcacagagatgaaggggccctgggggcagacagggataaggagagagggtgggagacagaagggaaagaggagagaagggagatgggaagtaaataagtgaagaggccaggagatgacgggaagagaagacagagtgaaaatggtcccgaatgcaccaaggagacagggaacgggaggagtaggggatgaacaaggcagggaagggtggggctgggtggggttgggcagatggggagccaagttggctggggctgtgtcccactcaccctgtgcagagctgacacagtctgaaaggacgagcctttcttggccttgcctttgcccttctcaatagctgcaggaaggagagtcaacaaaagacgatgaggtcaatgcaggcctgcaggtccatgccaaagtcaatgaatgtccactcgatgccctccttcttgtactcctcctgctccagcacaaacatgtggtggttgaagaactgctgcagcttctcgttggtgaagttgatgcagagctgctcaaagctgttgaactgcagggggcatgaggggtgggagcagtcagaaagtgggtgtgagtggccattggggctgtgcccgtccactgtgcctgagcccagcagggcgtggctggtcccctccatgtcaaggcagtgaaggagggcttcccctgaagacagagaaaatgactgcctctgtcaccacacagtccccactgccttcccatgtctggtccacagctggctctaagcaaatagctgttgaatgtgggagcgagtgagtgattgttctcccactcccaggggtcccaactcacatcgaagatctcgaagccagcgatgtccaggactcctatgaagtactggcatggctgcttggtctccagggtggcattgatgcgcgtcaccatccagttgaacatcctctcatacactgccttggccagtgccccagtggcatatatcacctgcaaggtggaggagagacccatattgagcagggttgttgggaagagtgaacttgaaaactctcatcccaccatgccagtctccctaccctgcccacccattatcatctgaagatggacccacctgctggacattctgccccttggtgacgtactcattgcccactttcacccgagggtggcacagccccttgagcaggtcggctgagttcagccccatgaggtaggcagacttgtcagcctctggaaggaaaaggcaagtagcaaagttggtaaagagatgactgctggccaggtgtggtggttcatgcctgtaatcccagcactttgggaggccaaggcaggcggatcacttgaggtcaggagtttgagaccaacctggccaacatgatgaaaccccaatccaaggatcaggaagtgtgagggtggtgtaggggatcataagagtgcacctattttcaaccctagcatctcaggcatctgggtcgtggagtggtgtgtacagcatcgatagaatccatattcccagactttcacaaaggtccttctgtcatcagacaaaatcctccaccttgaaccggttccagtcagtagataactgtactcagagctgagcctactaccttaacacccaacatggcacctccacgagcaagtatattgaccatagagcagaatccatgtccacctgtgtgaaggacactcagtgatgctctctcctgcttcctcagcccatgggcatcatgtccatcctggaagaggagtgcatgttccccaaggccaccgacatgaccttcaaggccaagctgtttgacaaccacctgggcaaatccgccaacttccagaagccacgcaatatcaaggggaagcctgaagcccacttctccctgatccactatgcccgcatcgtggactacaacatcattggctggctgcagaagaacaaggatcctctcaatgagactgtcgtgggcttgtatcagaagtcttccctcaagctgctcagcaccctgtttgccaactatgctggggctgatgcgcgtaagtagggactgaggctcccggtacagaggagcagggattctgccaaggttctgagccaggtcaattgctacaccccaccacttcaatgtcaggttgtaccccaaggtttacagactcagtgggatggaactgggtgaagaaactgaggcagccacattgaaggccctcacccaggggccaaatgccagcaaggatgtaaagaggggctgtgattctttactcacaccctacctccccacactgatgcttcttttgttgactctccttcctgcagctattgagaagggcaaaggcaaggccaagaaaggctcgtcctttcagactgtgtcagctctgcacagggtgagtgggacacagccacatgcaaggccatgggttgggaaacagaaaataagttagtgaacatgctcagggcatcacatgttggtaaattagctcaggcactggccagggaattgtgatttgcatgtagctggaccaggttatgccagtggttttgagaggtgaggctggagcatatgaggagggggattcagttccaggattagaagcctagactgggagcctaagccgggaagagactggtaaggcctcggtactggaagacgagataaggagaataaaaaaggagtgtaggatggaggagttgggtgtgcgggaaatggaaggagaagtacccaccccctcgtgtgcccccagattgcagatctgactcagaagatctttgaccttcgaggcaagtttaagcggcccaccctgcggagagtgaggatctctgcagatgccatgatgcaggcgctgctgggggcccgggctaaggagtccctggacctgcgggcccacctcaagcaggtgaaggaggacaccgagaaggtgagtgtgggctaaggccaggaaagaggatgctgaggggaagggctgtgggtgccaacaaccctaggcctgagggcagatggtgcttggagttggaggtagaagcagctagtaaggggtcctcagaaatgcaagaggaagacaggaagtagaaggggaagacaggaagtgcattagggctacaggaagtccatgtaagagcaaagaggtacatgaaggtccaggtgcagtggcttatgcctgtaatctttgaggtttaaaaaaaatttttttttaatttccttttttttttttttttgcgatggagtctctgctgcccaggctggagtgcaatgacaccatctcggttgctggagtgcagtgacaccatctcggctcactgcaacctctgcctcccaggatcaagtgattctcatgcctcagcctcccgagtagctgggactacaggtgcacaccaccatgttgttgttttaatttctacaaatatttttgggccatggtttacctcaggtaactgaaaccacacaaagtaaaattgcagaaaaggagggactactataataagaagagaaggaaggagacaggaagggcataaggcagacaggaagtggaggggaaagataggaagtgcaggaaggagacaggaagtggaggggaaagacaggaagtgcatgagggagacaggaagtggatggggaaagacagaaagtacatgagggagacaggaagtgctggggaaagacaggaagtgcatgagggggacaggaagtgcatgagggagacaggaagtgcatggggaaaattggcagggattatcttgaaaagacaggaagtgctccagaactagatacttaggcatccagggtagagtggccccacaggctggagggaagacagggattcttgagagactggagaccaagaagagaccctaacctctgactcatcgccatcctccaggaaaaccgggaggtgggagactggcacaagaacatcgatgcactgagtggaatggagggccgcaagaaaaagtttgagagctgagccttcctgcctactgcccctgccctgaggagggccctgaggaataaagcttctctctgagctgaaagtgactccatgtctattacccagggcttaggcaggagacagatgggaagactgcaggtggggctcccccaaagccacacagcaggttggggaccagatgggtctcccatgtgaagcactcttggctgtgttattgaaaagaatcccggggttcatgaatttggagagcggagctttgtttcttaagaagcggatcacaacctgaagaccagaagcatggcttcttgccaaaaaacaaaagcaggcactttaagggagggaagggcaaggcaggaatttatgctgagtgggttagctaagtgcacgtattcaactggttatagaaggagctatgaatattcatggacaggtggacacatggacacacgcatgtgtgagagacaatatcaatatcaacctaggaagtgctgggcattgtcttggctctgataatacatcagcaaacaagacagaaatgcctgcgtccttatgaacgtgttattttataagactctccagccctcatcccttccccagtgcagacttcgtgggaaccgaaggccccgtagctctcttcctgtgcagctgctgaaggcatttccagagcaacaggtcttccaggggcactcccagcttaaggggatgacgagacctcacatttgggaatcaggacctcattcaatcacgcagtcatttctcagtcagtggactcctgtgggccagcactgtgctgggagctaccctctcagaaagctccttgctgagcggagagaaagctgaactcacccataaagaccacaagcttcagcccagaatcagggtttccaatcctttcccctaatttgctttcttcctccctgctgtaaatcaggaagagagggctcgacgagaggaggagaacaggaggaaggctgaggatgaggcccggaagaagaaggctttgtccaacatgatgcattttgggggttacatccagaaggtaggtagggagcagcaggggttgccaggagatcctagtatagccctgaggaatgaggtgtccactgcagcaggtagactttaggtcaggtcccaggaagagattcccagctgctgtgggtggaagactgaggtctcctcatgcccagccctgagctggttttcagcctgaccgcggcttgcactaggaggggcttgctggggtagggggctacaggcagagcctggggcaccaatggtgccccccatgcctggctccagcagtgctcaggagcccccaaggaggctgggtgcagctggaagagccttgtgcctagagtcagagctctagttggagacccagctctgccacatacagttgtgtgaccttttgcaacctctgagcctcggtttcctcaactggcactcatattgcctgcttaagaataatggatcagaccttgaaagcattaatggctgcagaggataaggtactgatggctcgtgtggtttttaggtttaactgcaacccagacatctttcagcttccaatgcctcctggttcgtttggtataacgactgcaccttcacttcaccctctgctatttatatcttgccttaagtgctttcccttggtcctttatgctcctttgttttcccttcataaatgctctttgggcagccaaaaaaggagccaaattatcgcacttcaaagttgttggatttggtcaccctgccttctgctgttgcgaggttggggggcagtgttcctggaaaacctaaacattttaatacctgatgatttggctactttaaggcagcccttcgtctctaggactcagttttcattttttcccatccctctcctttttctctcctccttcctttggcttgtctcccaccctttctgcctctgatcgaaaacattagcaaatgtgccaagcttgaagaagaattgaaaactgtgacgaacaacttgaagtcactggaggctcaggctgagaaggtaggccaggaggatggtgtgggggaaaggcatcttttaagagctgctcaaaagaggccctgccagaaagcaacacttacagtagacattttagtaaaatggcaatattgtgaggtgatttttggagagttactagataacaaattcttttttttaactagagaatttattttatgttagggatatgaggcatcaatttaatttaaaccaagtgccaagtggataagttatcttgttgttatcccatgtaaaacaataggcaagaaagcagagaatgtattgcagtgtgccatttgatatcagaggttccattacctcctaagagatccttaacatctgttggctgagctggcgagttctttgcatgagaagccatgagtagattgagctgcagcctgacatctggaatgctctttctaattacagtactcgcaggcggccgc

SEQ ID NO: 5 - DNA, 22 bp, Artificial Sequence
  Description of Artificial Sequence: Synthetic primer
aaccaggaaatcttgggctata

SEQ ID NO: 6 - DNA, 19 bp, Artificial Sequence
  Description of Artificial Sequence: Synthetic primer
acacagatgtgtctccctg

SEQ ID NO: 7 - DNA, 18 bp, Artificial Sequence
  Description of Artificial Sequence: Synthetic probe
aggtcccctctctttacc

SEQ ID NO: 8 - DNA, 17 bp, Artificial Sequence
  Description of Artificial Sequence: Synthetic probe
tggcttccctccctctc

SEQ ID NO: 9 - DNA, 19 bp, Artificial Sequence
  Description of Artificial Sequence: Synthetic primer
taaggagtccctggacctg

SEQ ID NO: 10 - DNA, 18 bp, Artificial Sequence
  Description of Artificial Sequence: Synthetic primer
gccttagcccacactcac

SEQ ID NO: 11 - DNA, 12 bp, Artificial Sequence
  Description of Artificial Sequence: Synthetic probe
aggtgaaggagg

SEQ ID NO: 12 - DNA, 12 bp, Artificial Sequence
  Description of Artificial Sequence: Synthetic probe
aggtgaagaagg

SEQ ID NO: 13 - DNA, 15 bp, Homo sapiens
cttctacctcaaaaa

SEQ ID NO: 14 - DNA, 11 bp, Homo sapiens
gaagatactag

SEQ ID NO: 15 - DNA, 11 bp, Homo sapiens
taataacatta

SEQ ID NO: 16 - DNA, 16 bp, Homo sapiens
ggaattaagagaagca

SEQ ID NO: 17 - protein, 5 aa, Homo sapiens
ELREA

SEQ ID NO: 18 - DNA, 20 bp, Homo sapiens
ttcttctggggtcaggccag

SEQ ID NO: 19 - DNA, 19 bp, Homo sapiens
ctggcctgaccccagaaga

SEQ ID NO: 20 - DNA, 12 bp, Homo sapiens
actagtatcttc

SEQ ID NO: 21 - DNA, 11 bp, Homo sapiens
taatgttatta

SEQ ID NO: 22 - DNA, 41 bp, Homo sapiens
tgattcagactccccatcatgtgagtcatcagaacctaaca

SEQ ID NO: 23 - DNA, 40 bp, Homo sapiens
tgttaggttctgatgactcacatgatggggagtctgaatc

SEQ ID NO: 24 - DNA, 11 bp, Homo sapiens
gccacatggct

SEQ ID NO: 25 - DNA, 10 bp, Homo sapiens
agccatgtgg

SEQ ID NO: 26 - DNA, 226 bp, Homo sapiens
tgccgggcgcggtggctcacgcctgtaatcccagcactttgggaggccgaggcgggcggatcacgaggtcaggagatcgacaccatcccggctgaaacggtgaaaccccgtctctactaaaaatacaaaaaattagccgggcgtagtggcgggcgcctgtagtcccagctacttgggaggctgaggcaggagaatggcgtgaacccgggaggcggagcttgcagtg

SEQ ID NO: 27 - DNA, 12 bp, Homo sapiens
accgtgtggaag

SEQ ID NO: 28 - DNA, 343 bp, Homo sapiens
taatgaggacattatttttttttttttttttttttttttttttttttttttttttgagacggagtctcgctctgtcgcccaggccggactgtggactgcagtggcgcaatctcggctcactgcaagctccgcttcccgggttcacgccattctcctgcctcagcctcccgagtagctgggactacaggcgcccgccaccgcgcccggctaattttttgtatttttagtagagacggggtttcaccttgttagccaggatggtctcgatctcctgacctcatgatccacccgcctcggcctcccaaagtgctgggattacaggcgtgagccaccgcgcccggcc

SEQ ID NO: 29 - DNA, 11 bp, Homo sapiens
gaattatatct

SEQ ID NO: 30 - DNA, 25 bp, Homo sapiens
aggctccatgctgctccccgccgcc

SEQ ID NO: 31 - DNA, 13 bp, Homo sapiens
tgaaaggttcact

SEQ ID NO: 32 - DNA, 21 bp, Homo sapiens
gataaaaccctagccttcaaa

SEQ ID NO: 33 - DNA, 20 bp, Homo sapiens
ataaaaccctagccttcaaa

SEQ ID NO: 34 - DNA, 29 bp, Homo sapiens
tttcgatttgcagcaaattgacttcttta

SEQ ID NO: 35 - DNA, 20 bp, Homo sapiens
ttcaaaagggacatagaaaa

SEQ ID NO: 36 - DNA, 19 bp, Homo sapiens
tcaaaagggacatagaaaa

SEQ ID NO: 37 - DNA, 11 bp, Homo sapiens
gcaaataaaga

SEQ ID NO: 38 - DNA, 10 bp, Homo sapiens
taaagacaaa

SEQ ID NO: 39 - DNA, 29 bp, Homo sapiens
ggctactgcacaagctgcagcagctgccc

SEQ ID NO: 40 - DNA, 28 bp, Homo sapiens
gctactgcacaagctgcagcagctgccc